European Patent Specification EP 3 609 527 B1, published July 30, 2025. Title: Protein Conjugates. Applicant: TDW Group Almassy, Robert J. Brin, Elena Showalter, Richard E. Thomson, James A. The sequence listing filed with the application follows.

SEQUENCE LISTING (97 sequences)

SEQ ID NO: 1 - protein, 409 aa, Mycoplasma hominis
MSVFDSKFNGIHVYSEIGELETVLVHEPGREIDYITPARLDELLFSAILESHDARKEHQSFVKIMKDRGINVVELTDLVAETYDLASKAAKEEFIETFLEETVPVLTEANKKAVRAFLLSKPTHEMVEFMMSGITKYELGVESENELIVDPMPNLYFTRDPFASVGNGVTIHFMRYIVRRRETLFARFVFRNHPKLVKTPWYYDPAMKMPIEGGDVFIYNNETLVVGVSERTDLDTITLLAKNIKANKEVEFKRIVAINVPKWTNLMHLDTWLTMLDKNKFLYSPIANDVFKFWDYDLVNGGAEPQPQLNGLPLDKLLASIINKEPVLIPIGGAGATEMEIARETNFDGTNYLAIKPGLVIGYDRNEKTNAALKAAGITVLPFHGNQLSLGMGNARCMSMPLSRKDVKW

SEQ ID NO: 2 - protein, 409 aa, Artificial Sequence
  Mutated arginine deaminase
MSVFDSKFNGIHVYSEIGELETVLVHEPGREIDYITPARLDELLFSAILESHDARKEHQSFVKIMKDRGINVVELTDLVAETYDLASKAAKEEFIETFLEETVPVLTEANKEAVRAFLLSKPTHEMVEFMMSGITKYELGVESENELIVDPMPNLYFTRDPFASVGNGVTIHFMRYIVRRRETLFARFVFRNHPKLVKTPWYYDPAMKMSIEGGDVFIYNNETLVVGVSERTDLDTITLLAKNIKANKEVEFKRIVAINVPKWTNLMHLDTWLTMLDKNKFLYSPIANDVFKFWDYDLVNGGAEPQPQLNGLPLDKLLASIINKEPVLIPIGGAGATEMEIARETNFDGTNYLAIKPGLVIGYDRNEKTNAALKAAGITVLPFHGNQLSLGMGNARCMSMPLSRKDVKW

SEQ ID NO: 3 - protein, 392 aa, Mycoplasma phocicerebrale
IHVYSEIGELETVLVHEPGREIDYITPARLDELLFSAILESHDARKEHQSFVKQLKDNGINVVELTDLVAETFDLASKEEQEKLIEEFLEDSEPVLSEAHKTAVRKFLTSRKSTREMVEFMMAGITKYDLGIEADHELIVDPMPNLYFTRDPFASVGNGVTIHYMRYKVRQRETLFSRFVFSNHPKLVKTPWYYDPAMKMSIEGGDVFIYNNDTLVVGVSERTDLETITLLAKNIKANKEVEFKRIVAINVPKWTNLMHLDTWLTMLDKDKFLYSPIANDVFKFWDYDLVNGGAEPQPKENGLPLEGLLQSIINKKPVLIPIAGNNASHIDIERETHFDGTNYLAIKPGVVIGYARNEKTNAALAAAGIKVLPFHGNQLSLGMGNARCMSMP

SEQ ID NO: 4 - protein, 410 aa, Mycoplasma arginini
MSVFDSKFKGIHVYSEIGELESVLVHEPGREIDYITPARLDELLFSAILESHDARKEHKQFVAELKANDINVVELIDLVAETYDLASQEAKDKLIEEFLEDSEPVLSEEHKVVVRNFLKAKKTSRELVEIMMAGITKYDLGIEADHELIVDPMPNLYFTRDPFASVGNGVTIHYMRYKVRQRETLFSRFVFSNHPKLINTPWYYDPSLKLSIEGGDVFIYNNDTLVVGVSERTDLQTVTLLAKNIVANKECEFKRIVAINVPKWTNLMHLDTWLTMLDKDKFLYSPIANDVFKFWDYDLVNGGAEPQPVENGLPLEGLLQSIINKKPVLIPIAGEGASQMEIERETHFDGTNYLAIRPGVVIGYSRNEKTNAALEAAGIKVLPFHGNQLSLGMGNARCMSMPLSRKDVKW

SEQ ID NO: 5 - protein, 409 aa, Mycoplasma arthritidis
MSVFDSKFKGIHVYSEIGELETVLVHEPGKEIDYITPARLDELLFSAILESHDARKEHKEFVAELKKRGINVVELVDLIVETYDLASKEAKEKLLEEFLDDSVPVLSDEHRAAVKKFLQSQKSTRSLVEYMIAGITKHDLKIESDLELIVDPMPNLYFTRDPFASVGNGVTIHYMRYKVRQRETLFSRFVFSNHPKLVNTPWYYDPAEGLSIEGGDVFIYNNDTLVVGVSERTDLQTITLLAKNIKANKECEFKRIVAINVPKWTNLMHLDTWLTMLDKDKFLYSPIANDVFKFWDYDLVNGGDAPQPVDNGLPLEDLLKSIIGKKPTLIPIAGAGASQIDIERETHFDGTNYLAVAPGIVIGYARNEKTNAALEAAGITVLPFRGNQLSLGMGNARCMSMPLSRKDVK

SEQ ID NO: 6 - protein, 408 aa, Mycoplasma orale
  misc_feature (201)..(201): Xaa can be any naturally occurring amino acid
  misc_feature (263)..(263): Xaa can be any naturally occurring amino acid
  misc_feature (272)..(272): Xaa can be any naturally occurring amino acid
  misc_feature (294)..(294): Xaa can be any naturally occurring amino acid
SVFSDKFNGIHVYSEIGDLESVLVHEPGKEIDYITPARLDELLFSAILESTDARKEHKEFVEILKKQGINVVELVDLVVETYNLVDKKTQEKLLKDFLDDSEPVLSPEHRKAVEKFLKSLKSTKELIQYMMAGITKYDLGIKADKELIVDPMPNLYFTRDPFASVGNGVTIHYMRYKVRQRETLFSKFIFTNHPKLVKTPXYYDPAMKLSIEGGDVFIYNNDTLVVGVSERTDLETITLLAKNIKANKECEFKRIVAINVPKXTNLMHLDTXLTMLDKDKFLYSPIANDVFKFXDYDLVNGGSNPEPVVNGLPLDKLLESIINKKPVLIPIAGKGATEIETAVETHFDGTNYLAIKPGVVVGYSRNVKTNAALEANGIKVLPFKGNQLSLGMGNARCMSMPLSRKDVK

SEQ ID NO: 7 - protein, 391 aa, Mycoplasma gateae
IHVYSEIGELESVLVHEPGREIDYITPARLDELLFSAILESHDARKEHKLFVSELKANDINVVELTDLVTETYDLASQEAKDNLIEEFLEDSEPVLTEELKSVVRTYLKSIKSTRELIQMMMAGITKYDLGIEADHELIVDPMPNLYFTRDPFASVGNGVTIHYMRYKVRQRETLFSRFVFSNHPKLVNTPWYYDPSLKLSIEGGDVFIYNNNTLVVGVSERTDLETVTLLAKNIVANKECEFKRIVAINVPKWTNLMHLDTWLTMLDKDKFLYSPIANDVFKFWDYDLVNGGEEPQPVENGLPLEGLLESIINKKPILIPIAGEGASQIDIERETHFDGTNYLAIRPGVVIGYSRNEKTNAALEAAGIKVLPFHGNQLSLGMGNARCMSM

SEQ ID NO: 8 - protein, 392 aa, Mycoplasma phocidae
IHVYSEIGELQTVLVHEPGREIEYITPARLDELLFSAILESHDARKEHQEFVAELKKNNINVVELTDLVSETYDMVSKEKQEKLIEEFLEDSEPVLSEEHKGLVRKFLKSLKSSKELIQYMMAGITKHDLNIEADHELIVDPMPNLYFTRDPFASVGNGVTIHYMRYKVRQRETLFSRFIFANHPKLMNTPLYYNPDMKLSIEGGDVFVYNNETLVVGVSERTDLDTITLLAKNIKANKEREFKRIVAINVPKWTNLMHLDTWLTMLDKDKFLYSPIANDVFKFWDYDLVNGGDEPQPKVNGLPLEKLLESIINKKPILIPIAGTSASNIDVERETHFDGTNYLAIAPGVVIGYSRNVKTNEALEAAGIKVLPFKGNQLSLGMGNARCMSMP

SEQ ID NO: 9 - protein, 401 aa, Mycoplasma columbinum
MSKINVYSEIGELKEVLVHTPGDEIRRISPSRLDELLFSAILEPNEAIKEHKGFLKILQDKGIKVIQLSDLVAETYTYHATQKEREAFIEKWLDEAEPALTKDLRAKVKSYVLSKEGTPVAMVRTMMAGVSKQELNVESETELVVDPMPNLYFTRDPFASAGNGISLNNMKYVTRKRETIFAEFIFATHPDYKTTPHWFDRLDEGNIEGGDVFIYNKDTLVIGVSERTNKEAILTIAKKIKNNKEAKFKKIVAINVPPMPNLMHLDTWLTMVDKDKFLYSPNMLSVLKVWEIDLSKEIEMVETNKPLADVLESIIGVKPVLIPIAGKGATQLDIDIETHFDGTNYLTIAPGVVVGYSRNIKTEAALRAAGVTVLSFEGNQLSLGMGSARCMSMPLVREDVK

SEQ ID NO: 10 - protein, 407 aa, Mycoplasma iowae
MGNNIPKKINVFSEIGNLKRVLVHTPGKEIEYVTPQRLDELLFSAILDPVRAREEHKEFIKILESQGVEVVQLVDLTAETYDVAESQAKENFIQKWLDESLPKLTDENRNKVYSLLKSLEKDPKEMIRKMMSGVLASEIGVKSDVELIVDPMPNLYFTRDPFASVGNGITLHRMFRPTRRRETIFADFIFSNHPEYKSTQKYYEREDKFSLEGGDVFIYNNKTLVVGVSERTEKGAIKALAKAVQNNSNMSFEKIYAINVPKMSNLMHLDTWLTMLDTDKFLYSPNMMGVLKIWEIDLSDKSLKWKEIRDSLDHFLSTIIGKKAITVPVAGKDAMQFEIDIETHFDATNFIAVAPGVVIGYDRNKKTNEALKEAGIKVLSWNGDQLSLGMGSARCMTMPLYREELKK

SEQ ID NO: 11 - protein, 402 aa, Mycoplasma crocodyli
MNKINVYSEVGKLKEVLVHTPGDEIRRISPSRLEELLFSAILEPDSAIEEHKRFLKILEDNNIKVIQLDQLVADTYELVNPSVRDAFIEKWLNESEPKLDKKLREKVKEYLLHTQKTVGTKRMVRIMMAGVDRVELGVELDRQLVVDPMPNLYFTRDPFASAGNGISLNNMKYVTRKRETIFSEFIFENHPDYKTTPHWFDRLDKGNIEGGDVFIYNRTTLVIGISERTNKDALLTIANNIKSNKESKFERIVAVNVPPMPNLMHLDTWLTMVDHDKFLYSPNMMKTLKFWTIDLTKPIKMVELEESLSDMIETIIGKKPVLIPIAGHDASPLDVDIETHFDGTNYLTIAPGVVVGYSRNKLTEKALTKAGVKVLSFEGNQLSLGMGSARCMSMPLVREDIK

SEQ ID NO: 12 - protein, 430 aa, Mycoplasma fermentans
MQIIAKIDLLTNMLIFMKIYFIGRLIMKKINVYSEYGKLKEVLVHTPGDEIRRIAPSRLDELLFSAILEPDSAIAEHKRFVQLLKDNGIKVIQLDELFAKTFDLVSESVKQSLIERWLDECEPKLDATLRAKVKEYILELKAKSSKKMVRVMMAGIDKKELGIELDRDLVVDPMPNLYFTRDPFASVGNGISLHHMKYVTRQRETIFSEFIFDNNLDYNTVPRWFDRKDEGRIEGGDVFIYSADTLVVGVSERTNKEAINVMARKIAADKEVKFKRIYAINVPPMPNLMHLDTWLTMLDKNKFLYSPNMLSVLKVWRIDLNDPDFVWHEIEGSLEEILEQIIGMKPILIPIAGKGASQLDIDIETHFDGTNYLTIAPSVVVGYSRNEKTEKALKAAKVKVLSFEGNQLSLGMGSARCMSMPLIREDIKKK

SEQ ID NO: 13 - protein, 452 aa, Mycoplasma penetrans
MVITIALNILNKIYFKPQNRSILKLYRLPSLCTQISIFIGGKMSSIDKNSLGNGINVYSEIGELKEVLVHTPGDEIRYTAPSRLEELLFSAVLKADTAIEEHKGFVKILQNNGIKVIQLCDLVAETYELCSKEVRNSFIEQYLDEALPVLKKEIRPVVKDYLLSFPTVQMVRKMMSGILANELNIKQDNPLIIDGMPNLYFTRDPFASMGNGVSINCMKYPTRKREVIFSRFVFTNNPKYKNTPRYFDIVGNNGTIEGGDIFIYNSKTLVIGNSERTNFAAIESVAKNIQANKDCTFERIVVINVPPMPNLMHLDTWLTMLDYDKFLYSPNMMNVLKIWEIDLNVKPVKFVEKKGTLEEVLYSIIDKKPILIPIAGKGANQLDIDIETHFDGTNYLTIAPGVVVGYERNEKTQKALVEAGIKVLSFNGSQLSLGMGSARCMSMPLIRENLKK

SEQ ID NO: 14 - protein, 403 aa, Mycoplasma gallisepticum
MFNKIRVYSEIGKLRKVLVHTPGKELDYVTPQRLDELLFSSLLNPIKARQEHETFIKLLEDHDVECVQLSTLTAQTFQAVNSKIQEEFINRWLDECLPVLSEINRLKVYDYLKSLATNPQVMIRKMMSGILAKEVGIQSEVELVADPMPNLYFTRDPFASIGKGITLHSMFHPTRKRETIFADFIFSHHPEYKNAPKYYSREDKYSIEGGDLFVYDDKTLVIGVSERTEKKAIQSLAEKLRQNDETSFEKIYAINVPKMSNLMHLDTWLTMLDYDKFLYSPNMMGVLKIWEIDLIHPTLIWRELNESLEGFLSMVIGKKATLIPVAGEDSTQIEIDVETNFDATNFLVIQPGVVVGYDRNYKTNQALRDAGVKVISWNGDQLSLGMGSARCMSMPLYRDPIKK

SEQ ID NO: 15 - protein, 402 aa, Mycoplasma alligatoris
MSKINVYSEVGRLKEVLVHTPGDEIRRISPTRLEELLFSAILEPDTAIEEHKRFLNVLEKNGIKAIQLDELVAQTYDQVDQKIKDEFIDQWLQEAKPVLNDQLKKLVKNYLLKSQKEFSTKKMVRIMMAGIDKKEINIDLDRDLVVDPMPNLYFTRDPFASVGNGISLHNMKYQTRKRETIFAQFIFKYNKDYKTTPHWFDRFDHGSIEGGDVFVYTKDTLVIGISERTTKEAVLNIAKKIKANTDSKFKKIVAINVPPMPNLMHLDTWITMVDHDKFLYSPNMMKSLKFWLIDLSKEIKMVELEESLSNMLEAIIGKKPILIPIAGKNASQLDIDIETHFDGTNYLTIAPGVVVGYSRNKLTQKALEDAGVKVLSFDGNQLSLGMGSARCMSMPLVREDIK

SEQ ID NO: 16 - protein, 438 aa, Mycoplasma pneumoniae
MSKKQLVKTDGHNQLDQPNTKALQLKKKQFNSGVRVTSEISFLREVIAHHPGIETERVIDNQTFGSAMYLERAQKEHQLFIKILRQHGTKVHYLQDLLLEALSAADPNVRQDFIKNFLLESGIKSVSTFEACLNFFRSLDSLVDVIKVMFGGIKVSDVPPITPQRFADIHVSNSPFLIKPLSFSLYPHKFFNTLGTGVALFVTNDSELKRHSLVYEYIMRFHPRFDGVKLYTNRDFKNCLINSSDIIQISNEILLIGISHDTDVLGIESLARNLLSDHTNPIKQIIAINIHKFGAKTNLNKLIAMVDVDKFIIARKVLQATEIFELTATAQRDVDGLAQIKFKPLKFNFGEIIEAIIDKQPRFVIIGGGDEVAERKELLDCGMGVLNLSPGEIVVFDRNHYTNNLLNELGLIIHKIPASELSRGPSGPLEMVCSLWRE

SEQ ID NO: 17 - protein, 409 aa, Mycoplasma mobile
MKDTKDIINVFSEIGELKKVLIHTPGNELKYVSPYRLDELLFSNVLEWREAKKEHNEFIQKLKSEGVEPVELTDLVAESFEESSIKVKNDFIRQYLDEATPILDGLTKQKLLPFFLDIKHSTRKTIELMMSGITQKDISISHIERELIIDPMPNLYFSRDNFISIGNSVIISNMKYKTRKRETIFTDFIFKNHPLYKKVNMAFERKDLNNQISIIEGGDVLVYSKEILIIGISERTTMSAILELAENFKKTKRSFKKIYGVEVPKMKNLMHLDTWLTMIDYDKFIYSPNVLTDLKFWEINLDYEKISSKELHASLSEFLKLIIGKDPILIPIGGKGASQITIDIETNFVAANYLVIRPGVVIGYSRNYETQKALEGHGVKVIAFEGNQLSLGMGSSRCMSMPLIRSNLK

SEQ ID NO: 18 - protein, 411 aa, Streptococcus pyogenes
MTAQTPIHVYSEIGKLKKVLLHRPGKEIENLMPDYLERLLFDDIPFLEDAQKEHDAFAQALRDEGIEVLYLETLAAESLVTPEIREAFIDEYLSEANIRGRATKKAIRELLMAIEDNQELIEKTMAGVQKSELPEIPASEKGLTDLVESNYPFAIDPMPNLYFTRDPFATIGTGVSLNHMFSETRNRETLYGKYIFTHHPIYGGGKVPMVYDRNETTRIEGGDELVLSKDVLAVGISQRTDAASIEKLLVNIFKQNLGFKKVLAFEFANNRKFMHLDTVFTMVDYDKFTIHPEIEGDLRVYSVTYDNEELHIVEEKGDLAELLAANLGVEKVDLIRCGGDNLVAAGREQWNDGSNTLTIAPGVVVVYNRNTITNAILESKGLKLIKIHGSELVRGRGGPRCMSMPFEREDI

SEQ ID NO: 19 - protein, 408 aa, Enterococcus faecalis
MSHPINVFSEIGKLKTVMLHRPGKELENLMPDYLERLLFDDIPFLEKAQAEHDAFAELLRSKDIEVVYLEDLAAEALINEEVRRQFIDQFLEEANIRSESAKEKVRELMLEIDDNEELIQKAIAGIQKQELPKYEQEFLTDMVEADYPFIIDPMPNLYFTRDNFATMGHGISLNHMYSVTRQRETIFGQYIFDYHPRFAGKEVPRVYDRSESTRIEGGDELILSKEVVAIGISQRTDAASIEKIARNIFEQKLGFKNILAFDIGEHRKFMHLDTVFTMIDYDKFTIHPEIEGGLVVYSITEKADGDIQITKEKDTLDNILCKYLHLDNVQLIRCGAGNLTAAAREQWNDGSNTLAIAPGEVVVYDRNTITNKALEEAGVKLNYIPGSELVRGRGGPRCMSMPLYREDL

SEQ ID NO: 20 - protein, 403 aa, Mycoplasma capricolum
MEKKINVFSEIGTLKTVLVHRPGDEIENLTPELLERLLFDDVPFKDVAVKEHDAFTKIMRDNGVEVLYIEKLAAETLDQHPDLREKFIDQFISEANIEDKYKEKYRDFISSLDNYRMIKKMIAGTKKLELGIDEGYKAYPFIADPLPNVLFQRDPFSSVGFGITMNRMWSVTRNRETIFPDLVFKHHNRFANQVPYYYERDWKEETIEGGDILVLNKETLIIGVTQRTTLKAIEKFSERLFNDPESSYSKVIALDLPKSRAFMHLDTVFTNIDYDKFIAHPLIFDCIDEFKIYEVSKQGTKEVKKTLIELLSDAAGREVQIIRCGGNDVVGASREQWNDGTNVVALRPGKVIAYERNWITIDLLRKAGVEVLTIASSELSRGRGGPRCMTMPLWREDLQEIKR

SEQ ID NO: 21 - protein, 410 aa, Halothermothrix orenii
MFKKSPLNVTSEIGKLKKVLLHRPGHEIENLTPDLLERLLFDDIPYLKVAQEEHDAFAQTLRDNGVEVLYLHELAAEAIQEDEIRKKFIEQFLDEAGVIGKGARQVLKEYFADMDNETLIRKMMAGVRKKEIPAIEKVASLNDMVEEDYPFVLDPMPNLYFTRDPFATIGTGITLNHMRTETRNREVIFAEYIFSYHPDFKDTEIPFWFDRNETTSIEGGDELILSDKVLAMGISERTDAASIEKVARNIFTDGQPFETILAFKIPEKRAFMHLDTVFTMVDYDKFTIHAEIEGPLKVYSITKGDNDELKIDEEKATLEDTLKKYLGLDEVTLIRCAGGDYIDAGREQWNDGSNTLAIAPGEVVVYNRNHTTNRLLEEHGIKLHVIPSSELSRGRGGPRCMSMPLVREDI

SEQ ID NO: 22 - protein, 411 aa, Staphylococcus aureus
MTDGPIKVNSEIGALKTVLLKRPGKELENLVPDYLDGLLFDDIPYLEVAQKEHDHFAQVLREEGVEVLYLEKLAAESIENPQVRSEFIDDVLAESKKTILGHEEEIKALFATLSNQELVDKIMSGVRKEEINPKCTHLVEYMDDKYPFYLDPMPNLYFTRDPQASIGHGITINRMFWRARRRESIFIQYIVKHHPRFKDANIPIWLDRDCPFNIEGGDELVLSKDVLAIGVSERTSAQAIEKLARRIFENPQATFKKVVAIEIPTSRTFMHLDTVFTMIDYDKFTMHSAILKAEGNMNIFIIEYDDVNKDIAIKQSSHLKDTLEDVLGIDDIQFIPTGNGDVIDGAREQWNDGSNTLCIRPGVVVTYDRNYVSNDLLRQKGIKVIEISGSELVRGRGGPRCMSQPLFREDI

SEQ ID NO: 23 - protein, 417 aa, Pseudomonas plecoglossicida
MSAEKQKYGVHSEAGKLRKVMVCAPGLAHKRLTPSNCDELLFDDVIWVDQAKRDHFDFVTKMRERGVDVLEMHNLLTDIVQNPEALKWILDRKITPDTVGVGLTNEVRSWLEGQEPRHLAEFLIGGVAGQDLPESEGASVVKMYNDYLGHSSFILPPLPNTQFTRDTTCWIYGGVTLNPMYWPARRQETLLTTAIYKFHPEFTKADFQVWYGDPDQEHGQATLEGGDVMPIGKGIVLIGMGERTSRQAIGQLAQNLFAKGAVEQVIVAGLPKSRAAMHLDTVFSFCDRDLVTVFPEVVREIVPFIIRPDESKPYGMDVRRENKSFIEVVGEQLGVKLRVVETGGNSFAAEREQWDDGNNVVALEPGVVIGYDRNTYTNTLLRKAGIEVITISAGELGRGRGGGHCMTCPIVRDPINY

SEQ ID NO: 24 - protein, 417 aa, Pseudomonas putida
MSAEKQKYGVHSEAGKLRKVMVCAPGLAHKRLTPSNCDELLFDDVIWVDQAKRDHFDFVTKMRERGVDVLEMHNLLTDIVQNKDALKWILDRKITPDTVGVGLTNEVRSWLEGLEPRHLAEFLIGGVAGQDLPQSEGADVVKMYNDYLGHSSFILPPLPNTQFTRDTTCWIYGGVTLNPMYWPARRQETLLTTAIYKFHPQFTGADFQVWYGDPDKDHGNATLEGGDVMPIGKGIVLIGMGERTSRQAIGQLAQNLFAKGAVEKVIVAGLPKSRAAMHLDTVFSFCDRDLVTIFPEVVKEIVPFIIRPDESKPYGMDVRRENKSFIEVVGEQLGVKLRVVETGGNSFAAEREQWDDGNNVVAVEPGVVIGYDRNTYTNTLLRKAGIEVITISAGELGRGRGGGHCMTCPIVRDPIDY

SEQ ID NO: 25 - protein, 418 aa, Pseudomonas aeruginosa
MSTEKTKLGVHSEAGKLRKVMVCSPGLAHQRLTPSNCDELLFDDVIWVNQAKRDHFDFVTKMRERGIDVLEMHNLLTETIQNPEALKWILDRKITADSVGLGLTSELRSWLESLEPRKLAEYLIGGVAADDLPASEGANILKMYREYLGHSSFLLPPLPNTQFTRDTTCWIYGGVTLNPMYWPARRQETLLTTAIYKFHPEFANAEFEIWYGDPDKDHGSSTLEGGDVMPIGNGVVLIGMGERSSRQAIGQVAQSLFAKGAAERVIVAGLPKSRAAMHLDTVFSFCDRDLVTVFPEVVKEIVPFSLRPDASSPYGMSIRREEKTFLEVVAESLGLKKLRVVETGGNSFAAEREQWDDGNNVVCLEPGVVVGYDRNTYTNTLLRKAGVEVITISASELGRGRGGGHCMTCPIIRDPIDY

SEQ ID NO: 26 - protein, 402 aa, Mycobacterium tuberculosis complex
MGVELGSNSEVGALRVVILHRPGAELRRLTPRNTDQLLFDGLPWVSRAQDEHDEFAELLASRGAEVLLLSDLLTEALHHSGAARMQGIAAAVDAPRLGLPLAQELSAYLRSLDPGRLAHVLTAGMTFNELPSDTRTDVSLVLRMHHGGDFVIEPLPNLVFTRDSSIWIGPRVVIPSLALRARVREASLTDLIYAHHPRFTGVRRAYESRTAPVEGGDVLLLAPGVVAVGVGERTTPAGAEALARSLFDDDLAHTVLAVPIAQQRAQMHLDTVCTMVDTDTMVMYANVVDTLEAFTIQRTPDGVTIGDAAPFAEAAAKAMGIDKLRVIHTGMDPVVAEREQWDDGNNTLALAPGVVVAYERNVQTNARLQDAGIEVLTIAGSELGTGRGGPRCMSCPAARDPL

SEQ ID NO: 27 - protein, 409 aa, Mycoplasma arthritidis; identical to SEQ ID NO: 5

SEQ ID NO: 28 - protein, 410 aa, Artificial Sequence
  Artificial full length of Mycoplasma phocicerebrale
MSVFDSKFNGIHVYSEIGELETVLVHEPGREIDYITPARLDELLFSAILESHDARKEHQSFVKQLKDNGINVVELTDLVAETFDLASKEEQEKLIEEFLEDSEPVLSEAHKTAVRKFLTSRKSTREMVEFMMAGITKYDLGIEADHELIVDPMPNLYFTRDPFASVGNGVTIHYMRYKVRQRETLFSRFVFSNHPKLVKTPWYYDPAMKMSIEGGDVFIYNNDTLVVGVSERTDLETITLLAKNIKANKEVEFKRIVAINVPKWTNLMHLDTWLTMLDKDKFLYSPIANDVFKFWDYDLVNGGAEPQPKENGLPLEGLLQSIINKKPVLIPIAGNNASHIDIERETHFDGTNYLAIKPGVVIGYARNEKTNAALAAAGIKVLPFHGNQLSLGMGNARCMSMPLSRKDVKW

SEQ ID NO: 29 - protein, 410 aa, Artificial Sequence
  Artificial full length of Mycoplasma gateae
MSVFDSKFNGIHVYSEIGELESVLVHEPGREIDYITPARLDELLFSAILESHDARKEHKLFVSELKANDINVVELTDLVTETYDLASQEAKDNLIEEFLEDSEPVLTEELKSVVRTYLKSIKSTRELIQMMMAGITKYDLGIEADHELIVDPMPNLYFTRDPFASVGNGVTIHYMRYKVRQRETLFSRFVFSNHPKLVNTPWYYDPSLKLSIEGGDVFIYNNNTLVVGVSERTDLETVTLLAKNIVANKECEFKRIVAINVPKWTNLMHLDTWLTMLDKDKFLYSPIANDVFKFWDYDLVNGGEEPQPVENGLPLEGLLESIINKKPILIPIAGEGASQIDIERETHFDGTNYLAIRPGVVIGYSRNEKTNAALEAAGIKVLPFHGNQLSLGMGNARCMSMPLSRKDVKW

SEQ ID NO: 30 - protein, 410 aa, Artificial Sequence
  Artificial full length of Mycoplasma phocidae
MSVFDSKFNGIHVYSEIGELQTVLVHEPGREIEYITPARLDELLFSAILESHDARKEHQEFVAELKKNNINVVELTDLVSETYDMVSKEKQEKLIEEFLEDSEPVLSEEHKGLVRKFLKSLKSSKELIQYMMAGITKHDLNIEADHELIVDPMPNLYFTRDPFASVGNGVTIHYMRYKVRQRETLFSRFIFANHPKLMNTPLYYNPDMKLSIEGGDVFVYNNETLVVGVSERTDLDTITLLAKNIKANKEREFKRIVAINVPKWTNLMHLDTWLTMLDKDKFLYSPIANDVFKFWDYDLVNGGDEPQPKVNGLPLEKLLESIINKKPILIPIAGTSASNIDVERETHFDGTNYLAIAPGVVIGYSRNVKTNEALEAAGIKVLPFKGNQLSLGMGNARCMSMPLSRKDVKW

SEQ ID NO: 31 - protein, 410 aa, Mycoplasma salivarium
MSVFSSKFNGIHVYSEIGELETVLVHEPGKEIDYITPSRLDELLFSAILESHDARKEHQEFVATLKKEKINVVELTDLVTETYDLVDQKTKDKLIDEFLEDSEPVLTAELKATVKKFLKSFKETRKLIEVMMAGITKYDLGIKADRELIVDPMPNLYFTRDPFASVGNGVTIHYMRYKVRQRETLFSRFIFNNHPKLVKTPWYYDPAMKMSIEGGDVFIYNNDTLVVGVSERTDLDTITLLAKNIKANKECEFKRIVAINVPKWTNLMHLDTWLTMLDKDKFLYSPIANDIFKFWDYDLVNGGANPQPKDNGLPLDKLLKSIIGKEPVLIPIAGHHATEIEVARETHFDGTNYLAIRPGVVIGYARNEKTNEALKDAGITVLPFKGNQLSLGMGNARCMSMPLSRKDVKW

SEQ ID NO: 32 - protein, 411 aa, Mycoplasma spumans
MSVFDSKFKGIHVYSEIGELESVLVHEPGREIDYITPARLDELLFSAILESHDARKEHKGFVAELKKQNVNVIELTDLVAETYELASKEAQAKLIEDFIEDSEPVLNAEEAQAVRKFLSERKSTREMVEYMMSGLTKYELGLESADRELIVDPMPNLYFTRDPFASVGNGVTIHYMKYKVRQRETLFAKFVFSNHPKLVNTPRYYDPSMKLPIEGGDVFIYNNETLVVGCSERTELETITLLAKNIKANKEVEFKRIVAINVPKWTNLMHLDTWLTMLDKDKFLYSPIANDVFKFWDYDLVNGGEEPQPVENGLPLEELLASIINKKPTLIPIAGEGATHIDVERETHFDGTNYLAIAPALIIGYSRNEKTNAALEKAGITVLPFHGNQLSLGMGNARCMSMPLSRKDVKW

SEQ ID NO: 33 - protein, 410 aa, Mycoplasma auris
MSVFDSKFKGIHVYSEIGELETVLVHEPGREIDYITPKRLDELLFSAILESHEARKEHKQFVAELKANDINVVELTDLVAETYDLVSQELKDKLIEEFLDDSYPVLTEEHKKAVRSFLKSRSSTRELIEYMMAGITKYDLGIEAEGDLIVDPMPNLYFTRDPFASVGNGVTIHYMRYKVRQRETLFSRFIFDNHPKLVNTPRYYDPSLKLSIEGGDVFIYNNDTLVMGVSERTDLETVTLLAKNIVANKECEFKRIVAINVPHWTNLMHLDTWLTMLDKDKFLYSPIANDYFKFWDYDLVNGGAEPQPVVNELPLDKLLESIIHKKPILIPIAGEGASQIDLERETHFDGTNYLVLRPGVVVGYARNEKTNAALEAVGIKVLPFYGNQLSLGMGNSRCMSMPLSRKDVKW

SEQ ID NO: 34 - protein, 410 aa, Mycoplasma hyosynoviae
MSVFNSKFKGIHVYSEIGDLESVLVHEPGKEIDYITPSRLDELLFSAILESNDARKEHKEFVEILKKEGVNVVELVDLIAETIDLVDAKKKEALIDEYIEDSEPVVDAKVKPLVKKLLLGIKDTKELVKLMMAGITKYDLEIESEKELIIDPMPNLYFTRDPFASVGNGVTIHYMRYKVRQRETLFSRFVFRNHPKLTSTPWYYDPAMKLSIEGGDVFIYNNDTLVVGVSERTDLDTITLLAKNIKANKECEFKRIVAINVPKWTNLMHLDTWLTMLDKDKFLYSPIANDIFKFWDYDLVNGGSEPQPKDNGLPLEKLLESIIGKKPVLIPIAGCCASDIEIARETHFDGTNYLAIKPGVVIGYARNEKTNKALEKAGIKVLPFKGNQLSLGMGNARCMSMPLSRKDVKW

SEQ ID NO: 35 - protein, 409 aa, Mycoplasma cloacale
MSVFDKRFKGIHVYSEIGELQTVLVHEPGREIDYITPARLDELLFSAILESHDARKEHKEFVKILESQGINVVELTDLIAETYELASEEAKDNLIEEFLDESEPVLSEEHRILVRNFLKGITKTKELVKMMMAGITKYDLGIEADRELIVDPMPNLYFTRDPFASVGNGVTIHYMRYKVRQRETLFSRFIFENHPKLVSTPIYYHPSQGLSIEGGDVFIYNNDTLVVGVSERTDLQTITLLAKNIKANEECEFKRIVAINVPKWTNLMHLDTWLTMLDKNKFLYSPIANDVFKFWDYDLVNGGDEPQPVDNGLPLNELLASIIGEEPVLVPIAGEGASKMDIERETHFDGTNYLAIAPGVVVGYSRNEKTNAALEKAGIKVLPFKGHQLSLGMGNARCMSMPLYRKDVK

SEQ ID NO: 36 - protein, 412 aa, Mycoplasma alkalescens
MSVFDSKFKGIHVYSEIGELESVLVHEPGHEIDYITPSRLDELLFSAMLESHDARKEHKQFVAELKANNVNVIELTDLVAETYDLASQEAKDKLIEEFLEDSEPVLSEENKIAVRDFLKSRKTTRELIEVMMAGITKYDLGIKNCKCQDLVVDPMPNLYFTRDPFASVGNGITIHYMRYKVRQRETLFSRFIFANHPKLVNTPIYYHPSLKLSIEGGDVFIYNNDTLVVGVSERTDLETITLLAKNIVANKECEFKRIVAINVPKWTNLMHLDTWLTMLDKDKFLYSPIANDVFKFWDYDLVNGGAEPKPVENGSSLEAILESIIHKKPILIPIGGDSASQIEVERETHFDGTNYLAIRPGVVIGYSRNVKTNAALEAAGIKVIPFHGNQLSLGMGNARCMSMPLSRKDVKW

SEQ ID NO: 37 - protein, 401 aa, Mycoplasma iners
MSKINVYSEIGVLKEVLVHTPGDEIRRIAPSRLDELLFSAILEPSAAIQEHKSFLKILQDRGIKTIQLSDLVAETYKHYASEAEKEAFIEKYLDEATPVLSKDMRAKVKNYILSMQGEPVKMVRTMMAGVSKQELNVESEVELIVDPMPNLYFTRDPFASAGNGISLNNMKYVVRKRETIFAEFIFSIHPEYKKTPHWFDRLDNGSIEGGDVFIYNKDTLVIGVSERTNKEAIITIAKHIQDNKEAQFKKIVAINVPPMPNLMHLDTWLTMVDKNKFLYSPNMLSVLKVWEIDLSKPIEMVETNKPLAEVLESIIGEKPILIPIAGKDATQLDIDIETHFDGTNYLTIAPGVVVGYSRNVKTEAALRAAGVTVLSFEGNQLSLGMGSARCMSMPLVREDVK

SEQ ID NO: 38 - protein, 401 aa, Mycoplasma gallinarum
MSKIRVYSEIGNLKKVLVHTPGDEIRRISPSRLEELLFSAVLEPNAAIEEHKRFVKLLEDRGIQAIQLSDLVAETYVKYATAEQKAAFIEKYLDEATPALSAENRERAKKYILSLEMQPVKMIRTMMAGLSKYELNVESNIELIIDPMPNLYFTRDPFASAGNGISLNNMKYVVRKRETIFAEFIFAIHPEYKETPHWFDRLDHGSIEGGDVFVYNKDTLVIGVSERTNKEAIITIAKHIQDNKEAEFKKIVAINVPPMPNLMHLDTWLTMVDKNKFIYSPNMLSVLKIWEIDLAKPIEMVESNKSLTEVLESIIGEKPILIPIAGEGASQLDIDIETHFDGTNYLTIAPGVVVGYSRNEKTEKALKAAGITVLSFEGNQLSLGMGSARCMSMPLVREDVK

SEQ ID NO: 39 - protein, 405 aa, Mycoplasma pirum
MNSNQKGIHVYSEIGKLKEVLVHRPGRELDFLDPTRLDELLFAATLEAETARLEHDNFTNALKNQGVTVIELADLVAQTYSSSTPTIKAAFINKYLDEATPALTTKLRTLVKDFLTKQKSVRKMVDYMIGGILSTDLNIKGKPELIVEPMPNAYFTHDPFASVGNGVTLHYMKHNVRRREVLFSEFIFNNNERFQNTPRYIVPTKGLDIEGGDVFVYNKNTLVVGVSERTKMVTIKELAKNILKNKECLFKKIYAINVPKMPNLMHLDTWLTMLDHNKFLYSPNMLSVLKIWEIDISSGKSISSPKELNMDLSKALSIIIGKKPILIPVAGENASQIDINIETNFDATNYLVTQPGVVVGYSRNKKTEAALIKAGIEVIPFQGNQLSLGMGSARCMSMPLIREDV

SEQ ID NO: 40 - protein, 404 aa, Mycoplasma primatum
MSKSKINVYSEYGNLKEVLVHTPGDEIRRITPSRLDELLFSAILEPKSAIAEHKSFCQILKDNKVKAIQLDELVAATYKGVSESVQNSFVERWLDECEPKLENNVRPIVKEYLLKAAEQSVKKMIRIMMAGIDKREIGVESEVDFIVDPMPNLYFTRDPFASVGNGITLHHMKYVVRQRETLFSEFIFDNHPDYKFVPRYFDRDDEGKIEGGDVFIYNSKTLVVGISERTNKDAIRIVAKKIQANADAKFEKIFAINVPPMPNLMHLDTWLTMLDSNKFLYSPNMLSVLKVWEINLDDPALEWKEISGSLEEILTYIIGKKPILIPIAGKGASQFEIDIETHFDGTNYLAIAPSVVIGYSRNELTEKALKKAGVKVLSLDGNQLSLGMGSARCMSMPLIREDVK

SEQ ID NO: 41 - protein, 401 aa, Mycoplasma lipofaciens
MSKINVYSEVGVLKEVLVHTPGDEIRRVAPSRLDELLFSAILEPQDAIAEHKRFIKILEDNNIKVIQLDELVSETWEKATAEQRDAFIEKWLDEAEPVLDAKLRETVKKYLLSLNPVKKMVRTMMAGIDKKELKIELDRDLVVDPMPNLYFTRDPFASAGNGISLNNMKYVTRKRETIFAEFIFNIHPDYKTTPHWFDRLDKGNIEGGDVFIYNKDTLVLGVSERTNKDAVMTIAKHIQSNEQAKFKKLVAINVPPMPNLMHLDTWLTMVDHDKFLYSPNMLSVLKIWEIDLTPGKEIEMVESTKSLSDMLESIIGKKPVLIPIAGKDASQLDIDIETHFDGTNYLTIRPGVVVGYSRNCLTEQALKDAGVTVLSFDGNQLSLGMGSARCMSMPLVREDIK

SEQ ID NO: 42 - protein, 405 aa, Mycoplasma felifaucium
MNKINVYSEIGKLKEVLVHTPGNEIRRISPSRLDELLFSALLEPNFAAKEHTAFCEILKENGIKAIQLVDLVSDTWRIASEKAKTEFIERWLDECEPKLDSNLREIVRKHIYAIEKRSVKRMVKTMMAGIERRELPVTSKEVARELVVDPMPNLYFTRDPFASVGNGISLHHMKYVTRQRETIFAEFVFGNHPDYIDTPRWFDRSDDGRIEGGDVFIYGSKTLVIGVSERTNKEAIKVMAKKIQANKEATFEKIYAINVPPMPNLMHLDTWLTMLDKNKFLYSPNMLAVLQVWEIDLKDPELTWHELSGSLEEILHKIIGRKPILIPIAGHGAQQIDIDIETHFDGTNYLAIAPGVVVGYNRNVLTERALKKAGIKVLSFEGNQLSLGMGSARCMSMPLIRENLK

SEQ ID NO: 43 - protein, 404 aa, Mycoplasma imitans
MFNKIKVYSEIGRLRKVLVHTPGKELEYVTPQRLDELLFSSLLNPVKARQEHEAFIKILQDQGVECVQLTTLTAQTFQSATSEVKEKFINRWLDECLPKLSDDNRIKVYAYLKDLSSDPEVMIRKMMSGILAKEVNVQSDVELIADPMPNLYFTRDPFASIGKGVTLHSMFHPTRKRETIFADFVFSHHPEYKQTPKYYSRLNEYSIEGGDLFVYDDKTLVIGVSERTEKKAIQFLAEKLRENYETTFEKIYAINVPKMSNLMHLDTWLTMLDYDKFLYSPNMMGVLKIWEIDLTHEQLSWRELNESLEEFLSMVIGKKATTIPVAGEDSTQIEIDVETNFDATNFLVIQPGVVVGYDRNYKTNQALVNAGIKVLSWNGDQLSLGMGSARCMSMPLYRDPIKKG

SEQ ID NO: 44 - protein, 401 aa, Mycoplasma opalescens
MSKINVYSEIGTLKEVLVHTPGDEIRRVAPARLDELLFSAILEPNHAIAEHKAFIKILEDNGIKVIQLDELVVQTWNQVDEATRKAFVTKWLDECEPKLESNVRVEVEKYIYSLAKEPKKMVRTMMAGISKEELPLNVNRPLVVDPMPNLYFTRDPFASVGTGISLHHMKYVTRQRETIFAQFVFDNHKDYNTVPRWFDNKDQGRIEGGDVFIYNTKTLVIGVSERTDKDAIKIMAKKIQADKNCKFEKIFAINVPPMPNLMHLDTWLTMVDRNKFLYSPNMLSVLKVWEIDLKDASLAWKEIEGSLSQILEKIIGEKPILIPIAGENASQLDIDIETHFDGTNYLTIAPGVVVGYSRNVKTEQALKAAGVKVLSFEGNQLSLGMGSARCMSMPLIREDLK

SEQ ID NO: 45 - protein, 425 aa, Mycoplasma moatsii
MKKNAINVYSEIGKLKKVLVHRPGDELKYVTPQRMDELLMSAIIELEQAKEEHDAFTKILRDNGVEVIELADLTAEMYDSLTPSEKDAFLNQWVKEASWGKKSSIDALKIKKNLSKKVFDYVKSIKPTRKMIDKLMAGVLLSEIGEKSIILNKDKKNEMVIDLVVDPMPNLYFTRDPFASVGNGITLHNMKYPTRKRETIFAQWIFNKHPEYKDVPQFISKRDGKETIEGGDVFIYTKDVLAIGVSERTNMEAILRIATNIKKDKNCEFKKIVAINVPPMGNLMHLDTWLTMLDKDLFLYSGNIKSALKVWEIDLTKPITPKSPKLSTAKLADILAKIVGKKVRMIPIGGKDGNQMDIDIETHFDGTNYLAIAPGVVVGYHRNRKTQKALEEAGVKVLAFQGNQLSLGMGSARCMSMPLVREEVK

SEQ ID NO: 46 - protein, 399 aa, Mycoplasma elephantis
MSQINVFSEIGQLKEVLVHTPGDEIRRISPKRYNELLFSAILEADVAIKEHKSFVKILEENNVKVIQLKDILLETWNICSKEAKNIFINKWIEEAQPVIHSSSLKEKIKLFLKSKTPLEIIDIMMKGILKQELGIEYKHELIIDPMPNLYFTRDPFTSMGSGITINNMKYQTRKRETIFSEFIFNNHPKYKNTPRWFDRFDSGNIEGGDLFVYTKETIVVGVSERTKKKAILKIAKNIQENNNSFKKIVVIKVPIMQNLMHLDTWIVMVDFDKFIYSPNVTKSLKFWEIDLTKKPKFIQLKNETLEDVLYRVIGKKPILIPVAGENANQIDIDVETHFDATNYLTIRPGVVVGYSRNKKTEEALINAGVKVYAFEGNQLSLGMGSARCMSMPLIREDII

SEQ ID NO: 47 - protein, 399 aa, Mycoplasma testudinis
MKNINVYSEVGKLKEVVVHTPGEELHNVAPSRLQELLTSAVLEPEVARKEHLKFIKILNDYGVKVIQIVDLITETYEAVDSNKKEAFINNWLDNSVPKLTDKNRMILRNYLTQFSTKAMIRKMISGIRAKELNLKTPSALLVDPMPNLCFARDTFACVGSAISLSTMKHPTRRREALLTEFIFQNHPKYKDVIKYFDSKNSKATIEGGDIFVYNPKTLVVGNSERTNMQACLLLAKKIQSNPNNKFEKIVIVNVPPLPHLMHLDTWLTMVDYDKFIYSPNILHTLKFWVIDLKKRKLEAVEKHNTLKAMLRMIIKKEPILIPVGDVGADQLDIDLETHFDATNYLALAPGVVVGYDRNIKTQRALEKAGVKVLSFSGNQLSLAMGSARCLSMPLIREEN

SEQ ID NO: 48 - protein, 410 aa, Mycoplasma canadense
MSVFDSKFKGIHVYSEIGELESVLVHEPGREIDYITPARLDELLFSAILESHDARKEHKQFVSELKANDINVVELTDLVAETYDLASQEAKDKLIEEFLEDSEPVLSEEHKAIVRKYLKGIQPTRKLIEMMMAGITKYDLGIEADHELIVDPMPNLYFTRDPFASVGNGVTIHYMRYKVRQRETLFSRFVFSNHPKLVNTPWYYDPSLKLSIEGGDVFVYNNDTLVVGVSERTDLQTVTLLAKNIVANKECEFKRIVAINVPKWTNLMHLDTWLTMLDKDKFLYSPIANDVFKFWDYDLVNGGSEPQPVENGLPLEGLLESIINKKPILIPIAGEGASQMEIERETHFDGTNYLAIRPGVVIGYSRNEKTNAALEAAGIKVLPFHGNQLSLGMGNARCMSMPLSRKDVKW

SEQ ID NO: 49 - protein, 409 aa, Mycoplasma anseris
MSVFDKRFKGIHVYSEIGELQTVLVHEPGREIDYITPARLDELLFSAILESHDARAEHKKFVATLKEQGINTVELTDLVAETYDLASQEARDNLLEEFLDDSAPVLSEEHKEIVRTYLKGIKGTRKLIETMMAGITKYDLGIEAEQELIVDPMPNLYFTRDPFASVGNGVTIHYMRYKVRQRETLFSRFIFSNHPQLVNTPWYYNPAEGLSIEGGDVFIYNNDTLVVGVSERTDLQTITLLAKNIKANEECEFKRIVAINVPKWTNLMHLDTWLTMLDTNKFLYSPIANDVFKFWDYDLVNGGDEPQPVDNGLPLNELLKSIIGEEPILIPIAGDGATQIEIERETHFDGTNYLAIAPGVVIGYSRNEKTNAALEAAGIKVLPFKGHQLSLGMGNARCMSMPLYRKDVK

SEQ ID NO: 50 - protein, 401 aa, Mycoplasma meleagridis
MSKINVYSEIGVLKEVLVHTPGDEIRRISPSRLDELLFSAILQPEQAIKEHQSFVKILQDRGIKVIQLSDLVAETYVKYATSKEKESFIEKWLDEATPALNSENRARVKNYITAMQGQPVKMVRAMMAGVSKQELNIESDVELIVDPMPNLYFTRDPFASAGNGISLNNMKYVVRKRETIFAEFIFSIHPEYKQTPHWFDRLDKGNIEGGDVFIYNKDTLVIGVSERTNKEAILTIAEHIKNNKEAKFKKIVAINVPPMPNLMHLDTWLTMVDKNKFLYSPNMLSVLKIWEIDLSKEIKMVETSKPLADVLESIIGEKPILIPIAGENASQLDIDIETHFDGTNYLTIAPGVVVGYSRNVKTEAALKAAGVTVYSFDGNQLSLGMGSGRCMSMPLVREDVK

SEQ ID NO: 51 - protein, 404 aa, Mycoplasma alvi
MSIKENGIHVYSEIGKLRDVLVHRPGRELNFLDPSRLDELLFAATLEPETARLEHDNFTTVLKNQGVNVIELADLVSQTYSKVDSKVKKEFIDQYLNEATPKLTSELSKKVYDFLTKQKSNREMVDFMMGGILSSDLNIKGQPYLIVEPMPNLYFTRDPFASVGNGATIHWMKHNVRRREVLFANFIFKYNERFQNTPKYITPTKGLDIEGGDVFVYNKKTLVVGVSERTKMETIKELAKNISKNKECTFTKIYAINVPKMPNLMHLDTWLTMLDYNKFLYSPNMLSVLKVWEINISNNKVSAPKELNVNLEKALSMIIGKKPILIPVAGANASQIDINIETNFDATNYLVIEPGVVVGYSRNKKTEEALVKAGIKVLPFHGNQLSLGMGSARCMSMPLYREDV

SEQ ID NO: 52 - protein, 410 aa, Mycoplasma penetrans
MSSIDKNSLGNGINVYSEIGELKEVLVHTPGDEIRYTAPSRLEELLFSAVLKADTAIEEHKGFVKILQNNGIKVIQLCDLVAETYELCSKEVRNSFIEQYLDEALPVLKKEIRPVVKDYLLSFPTVQMVRKMMSGILANELNIKQDNPLIIDGMPNLYFTRDPFASMGNGVSINCMKYPTRKREVIFSRFVFTNNPKYKNTPRYFDIVGNNGTIEGGDIFIYNSKTLVIGNSERTNFAAIESVAKNIQANKDCTFERIVVINVPPMPNLMHLDTWLTMLDYDKFLYSPNMMNVLKIWEIDLNVKPVKFVEKKGTLEEVLYSIIDKKPILIPIAGKGANQLDIDIETHFDGTNYLTIAPGVVVGYERNEKTQKALVEAGIKVLSFNGSQLSLGMGSARCMSMPLIRENLKK

SEQ ID NO: 53 - protein, 404 aa, Mycoplasma fermentans
MKKINVYSEYGKLKEVLVHTPGDEIRRIAPSRLDELLFSAILEPDSAIAEHKRFVQLLKDNGIKVIQLDELFAKTFDLVSESVKQSFIERWLDECEPKLDATLRAKVKEYILELKAKSSKKMVRVMMAGIDKKELGIELDRDLVVDPMPNLYFTRDPFASVGNGISLHHMKYVTRQRETIFSEFIFDNNLDYNTVPRWFDRKDEGRIEGGDVFIYSADTLVVGVSERTNKEAINVMARKIAADKEVKFKRIYAINVPPMPNLMHLDTWLTMLDKNKFLYSPNMLSVLKVWRIDLNDPDFVWHEIEGSLEEILEQIIGMKPILIPIAGKGASQLDIDIETHFDGTNYLTIAPSVVVGYSRNEKTEKALKAAKVKVLSFEGNQLSLGMGSARCMSMPLIREDIKKK

SEQ ID NO: 54 - protein, 404 aa, Mycoplasma pneumoniae
MKYNINVHSEIGQLQTVLVHTPGNEIRRISPRRLDDLLFSAVIEPDTAIQEHQTFCQLLQEQNIEVVQLTDLTATTFDKANATAQNQFIETWLDQAEPKLTPEHRKVAKQYLLEQKAKSTLSMVRSMMGGIDKRKVAAANTINGDFLVDPMPNLYFTRDPFASIGHGISINRMKYLTRRRETLFASFIFANHPIIAARKFYFKPIDMGTIEGGDIFVYDQQTVVMGLSERTTEAAINVLAKKIQQDSSTSFKRIFVINVPQLPNLMHLDTWLTMLDRNKFLYSPNMLAVLKAWRIDFTDPALKWNEIAGDLSTILHTIIGQKPMLIPIAGADANQTEIDIETHFDGTNYLTIAPSVVVGYARNKLTHQTLEAAGVKVIAFKGNQLSLGMGSARCMSMPLVRKPL

SEQ ID NO: 55 - protein, 414 aa, Mycoplasma sp. CAG:877
MEKIHVTSEIGPLKKVLLHRPGNELLNLTPDTLSRLLFDDIPYLPDAIKEHDEFADALRANGVEVVYLENLMADVLDLSDEIRDKFIKQFIYEAGIRTPKYKYLVFDYLDQITNSKKLVLKTMEGIQISDIPRRKREIEKSLVDLIETEDEFIADPMPNLYFTRDPFASVGEGISLNKMYSVTRNRETIYAEYIFKYHPDYKDQARLYYDRYNPYHIEGGDVLNINDHVLAIGISQRTTAEAIDQIAKNLFKDPECKIDTILAFNIPESRAFMHLDTVFTQVDYDKFTYHPGIMGTLQVFEITEGDDPNSDEDLTVTEINAPLEEILTKYVGRKVTLIPCAGGDKVSAEREQWNDGSNTLCIAPGVVVVYDRNNLTNAVLRSYGLKVIEIHGAELSRGRGGPRCMSMPLVREDI

SEQ ID NO: 56 - protein, 408 aa, Mycoplasma sp. CAG:472
MHVTSEIKKLKKVLVHRPGKELLNLTPDTLGRLLFDDIPYLKDAILEHDEFCQILRDNDVEVVYLEDLMAETLDENPQVKPSFIRQFIYEAGVRTPKYKDLLFDYLMSYTNNKELVLKTMEGIKVSEVHRNKQDSEYSLVDQISEETKFLAEPMPNLYFTRDPFASVGDGIILNKMHSVTRSRETIYAYYIFNYHPDYMDKVPKYYDRENPFSIEGGDVLNLNEHTLAIGISQRTSAEAIDLVAKNMFNDEKCNIDTILAFKIPECRAFMHLDTVFTQIDIDKFTYHPGIMDTLEVFEITKNEDDLDEVRVIKKEGSLENILEEYLGIDITLIPCAGGDKIASEREQWNDGTNTLCIAPGVVVVYNRNNITNEVLREKGIKVIEMNSAELSRGRGGPRCMSMPLERED

SEQ ID NO: 57 - protein, 401 aa, Artificial Sequence
  Made in Lab - M. columbinum - M. gallinarum chimeric ADI
MSKINVYSEIGELKEVLVHTPGDEIRRISPSRLDELLFSAILEPNEAIKEHKGFLKILQDKGIKVIQLSDLVAETYVKYATAEQKAAFIEKYLDEATPALSAENRERAKKYILSLEMQPVKMIRTMMAGLSKYELNVESNIELIIDPMPNLYFTRDPFASAGNGISLNNMKYVTRKRETIFAEFIFATHPDYKTTPHWFDRLDEGNIEGGDVFIYNKDTLVIGVSERTNKEAILTIAKKIKNNKEAKFKKIVAINVPPMPNLMHLDTWLTMVDKDKFLYSPNMLSVLKVWEIDLSKEIEMVETNKPLADVLESIIGVKPVLIPIAGKGATQLDIDIETHFDGTNYLTIAPGVVVGYSRNIKTEAALRAAGVTVLSFEGNQLSLGMGSARCMSMPLVREDVK

SEQ ID NO: 58 - protein, 401 aa, Artificial Sequence
  Made in Lab - M. columbinum - M. iners chimeric ADI
MSKINVYSEIGELKEVLVHTPGDEIRRISPSRLDELLFSAILEPNEAIKEHKGFLKILQDKGIKVIQLSDLVAETYKHYASEAEKEAFIEKYLDEATPVLSKDMRAKVKNYILSMQGEPVKMVRTMMAGVSKQELNVESEVELIVDPMPNLYFTRDPFASAGNGISLNNMKYVTRKRETIFAEFIFATHPDYKTTPHWFDRLDEGNIEGGDVFIYNKDTLVIGVSERTNKEAILTIAKKIKNNKEAKFKKIVAINVPPMPNLMHLDTWLTMVDKDKFLYSPNMLSVLKVWEIDLSKEIEMVETNKPLADVLESIIGVKPVLIPIAGKGATQLDIDIETHFDGTNYLTIAPGVVVGYSRNIKTEAALRAAGVTVLSFEGNQLSLGMGSARCMSMPLVREDVK

SEQ ID NO: 59 - protein, 401 aa, Artificial Sequence
  Made in Lab - M. columbinum - M. meleagridis chimeric ADI
MSKINVYSEIGELKEVLVHTPGDEIRRISPSRLDELLFSAILEPNEAIKEHKGFLKILQDKGIKVIQLSDLVAETYVKYATSKEKESFIEKWLDEATPALNSENRARVKNYITAMQGQPVKMVRAMMAGVSKQELNIESDVELIVDPMPNLYFTRDPFASAGNGISLNNMKYVTRKRETIFAEFIFATHPDYKTTPHWFDRLDEGNIEGGDVFIYNKDTLVIGVSERTNKEAILTIAKKIKNNKEAKFKKIVAINVPPMPNLMHLDTWLTMVDKDKFLYSPNMLSVLKVWEIDLSKEIEMVETNKPLADVLESIIGVKPVLIPIAGKGATQLDIDIETHFDGTNYLTIAPGVVVGYSRNIKTEAALRAAGVTVLSFEGNQLSLGMGSARCMSMPLVREDVK

SEQ ID NO: 60 - protein, 401 aa, Artificial Sequence
  Made in Lab - M. gallinarum - M. columbinum chimeric ADI
MSKIRVYSEIGNLKKVLVHTPGDEIRRISPSRLEELLFSAVLEPNAAIEEHKRFVKLLEDRGIQAIQLSDLVAETYTYHATQKEREAFIEKWLDEAEPALTKDLRAKVKSYVLSKEGTPVAMVRTMMAGVSKQELNVESETELVVDPMPNLYFTRDPFASAGNGISLNNMKYVVRKRETIFAEFIFAIHPEYKETPHWFDRLDHGSIEGGDVFVYNKDTLVIGVSERTNKEAIITIAKHIQDNKEAEFKKIVAINVPPMPNLMHLDTWLTMVDKNKFIYSPNMLSVLKIWEIDLAKPIEMVESNKSLTEVLESIIGEKPILIPIAGEGASQLDIDIETHFDGTNYLTIAPGVVVGYSRNEKTEKALKAAGITVLSFEGNQLSLGMGSARCMSMPLVREDVK

SEQ ID NO: 61 - protein, 401 aa, Artificial Sequence
  Made in Lab - M. gallinarum - M. iners chimeric ADI
MSKIRVYSEIGNLKKVLVHTPGDEIRRISPSRLEELLFSAVLEPNAAIEEHKRFVKLLEDRGIQAIQLSDLVAETYKHYASEAEKEAFIEKYLDEATPVLSKDMRAKVKNYILSMQGEPVKMVRTMMAGVSKQELNVESEVELIVDPMPNLYFTRDPFASAGNGISLNNMKYVVRKRETIFAEFIFAIHPEYKETPHWFDRLDHGSIEGGDVFVYNKDTLVIGVSERTNKEAIITIAKHIQDNKEAEFKKIVAINVPPMPNLMHLDTWLTMVDKNKFIYSPNMLSVLKIWEIDLAKPIEMVESNKSLTEVLESIIGEKPILIPIAGEGASQLDIDIETHFDGTNYLTIAPGVVVGYSRNEKTEKALKAAGITVLSFEGNQLSLGMGSARCMSMPLVREDVK

SEQ ID NO: 62 - protein, 401 aa, Artificial Sequence
  Made in Lab - M. gallinarum - M. meleagridis chimeric ADI
MSKIRVYSEIGNLKKVLVHTPGDEIRRISPSRLEELLFSAVLEPNAAIEEHKRFVKLLEDRGIQAIQLSDLVAETYVKYATSKEKESFIEKWLDEATPALNSENRARVKNYITAMQGQPVKMVRAMMAGVSKQELNIESDVELIVDPMPNLYFTRDPFASAGNGISLNNMKYVVRKRETIFAEFIFAIHPEYKETPHWFDRLDHGSIEGGDVFVYNKDTLVIGVSERTNKEAIITIAKHIQDNKEAEFKKIVAINVPPMPNLMHLDTWLTMVDKNKFIYSPNMLSVLKIWEIDLAKPIEMVESNKSLTEVLESIIGEKPILIPIAGEGASQLDIDIETHFDGTNYLTIAPGVVVGYSRNEKTEKALKAAGITVLSFEGNQLSLGMGSARCMSMPLVREDVK

SEQ ID NO: 63 - protein, 401 aa, Artificial Sequence
  Made in Lab - M. iners - M. columbinum chimeric ADI
MSKINVYSEIGVLKEVLVHTPGDEIRRIAPSRLDELLFSAILEPSAAIQEHKSFLKILQDRGIKTIQLSDLVAETYTYHATQKEREAFIEKWLDEAEPALTKDLRAKVKSYVLSKEGTPVAMVRTMMAGVSKQELNVESETELVVDPMPNLYFTRDPFASAGNGISLNNMKYVVRKRETIFAEFIFSIHPEYKKTPHWFDRLDNGSIEGGDVFIYNKDTLVIGVSERTNKEAIITIAKHIQDNKEAQFKKIVAINVPPMPNLMHLDTWLTMVDKNKFLYSPNMLSVLKVWEIDLSKPIEMVETNKPLAEVLESIIGEKPILIPIAGKDATQLDIDIETHFDGTNYLTIAPGVVVGYSRNVKTEAALRAAGVTVLSFEGNQLSLGMGSARCMSMPLVREDVK

SEQ ID NO: 64 - protein, 401 aa, Artificial Sequence
  Made in Lab - M. iners - M. gallinarum chimeric ADI
MSKINVYSEIGVLKEVLVHTPGDEIRRIAPSRLDELLFSAILEPSAAIQEHKSFLKILQDRGIKTIQLSDLVAETYVKYATAEQKAAFIEKYLDEATPALSAENRERAKKYILSLEMQPVKMIRTMMAGLSKYELNVESNIELIIDPMPNLYFTRDPFASAGNGISLNNMKYVVRKRETIFAEFIFSIHPEYKKTPHWFDRLDNGSIEGGDVFIYNKDTLVIGVSERTNKEAIITIAKHIQDNKEAQFKKIVAINVPPMPNLMHLDTWLTMVDKNKFLYSPNMLSVLKVWEIDLSKPIEMVETNKPLAEVLESIIGEKPILIPIAGKDATQLDIDIETHFDGTNYLTIAPGVVVGYSRNVKTEAALRAAGVTVLSFEGNQLSLGMGSARCMSMPLVREDVK

SEQ ID NO: 65 - protein, 401 aa, Artificial Sequence
  Made in Lab - M. iners - M. meleagridis chimeric ADI
MSKINVYSEIGVLKEVLVHTPGDEIRRIAPSRLDELLFSAILEPSAAIQEHKSFLKILQDRGIKTIQLSDLVAETYVKYATSKEKESFIEKWLDEATPALNSENRARVKNYITAMQGQPVKMVRAMMAGVSKQELNIESDVELIVDPMPNLYFTRDPFASAGNGISLNNMKYVVRKRETIFAEFIFSIHPEYKKTPHWFDRLDNGSIEGGDVFIYNKDTLVIGVSERTNKEAIITIAKHIQDNKEAQFKKIVAINVPPMPNLMHLDTWLTMVDKNKFLYSPNMLSVLKVWEIDLSKPIEMVETNKPLAEVLESIIGEKPILIPIAGKDATQLDIDIETHFDGTNYLTIAPGVVVGYSRNVKTEAALRAAGVTVLSFEGNQLSLGMGSARCMSMPLVREDVK

SEQ ID NO: 66 - protein, 401 aa, Artificial Sequence
  Made in Lab - M. meleagridis - M. columbinum chimeric ADI
MSKINVYSEIGVLKEVLVHTPGDEIRRISPSRLDELLFSAILQPEQAIKEHQSFVKILQDRGIKVIQLSDLVAETYTYHATQKEREAFIEKWLDEAEPALTKDLRAKVKSYVLSKEGTPVAMVRTMMAGVSKQELNVESETELVVDPMPNLYFTRDPFASAGNGISLNNMKYVVRKRETIFAEFIFSIHPEYKQTPHWFDRLDKGNIEGGDVFIYNKDTLVIGVSERTNKEAILTIAEHIKNNKEAKFKKIVAINVPPMPNLMHLDTWLTMVDKNKFLYSPNMLSVLKIWEIDLSKEIKMVETSKPLADVLESIIGEKPILIPIAGENASQLDIDIETHFDGTNYLTIAPGVVVGYSRNVKTEAALKAAGVTVYSFDGNQLSLGMGSGRCMSMPLVREDVK

SEQ ID NO: 67 - protein, 401 aa, Artificial Sequence
  Made in Lab - M. meleagridis - M. gallinarum chimeric ADI
MSKINVYSEIGVLKEVLVHTPGDEIRRISPSRLDELLFSAILQPEQAIKEHQSFVKILQDRGIKVIQLSDLVAETYVKYATAEQKAAFIEKYLDEATPALSAENRERAKKYILSLEMQPVKMIRTMMAGLSKYELNVESNIELIIDPMPNLYFTRDPFASAGNGISLNNMKYVVRKRETIFAEFIFSIHPEYKQTPHWFDRLDKGNIEGGDVFIYNKDTLVIGVSERTNKEAILTIAEHIKNNKEAKFKKIVAINVPPMPNLMHLDTWLTMVDKNKFLYSPNMLSVLKIWEIDLSKEIKMVETSKPLADVLESIIGEKPILIPIAGENASQLDIDIETHFDGTNYLTIAPGVVVGYSRNVKTEAALKAAGVTVYSFDGNQLSLGMGSGRCMSMPLVREDVK

SEQ ID NO: 68 - protein, 401 aa, Artificial Sequence
  Made in Lab - M. meleagridis - M. iners chimeric ADI
MSKINVYSEIGVLKEVLVHTPGDEIRRISPSRLDELLFSAILQPEQAIKEHQSFVKILQDRGIKVIQLSDLVAETYKHYASEAEKEAFIEKYLDEATPVLSKDMRAKVKNYILSMQGEPVKMVRTMMAGVSKQELNVESEVELIVDPMPNLYFTRDPFASAGNGISLNNMKYVVRKRETIFAEFIFSIHPEYKQTPHWFDRLDKGNIEGGDVFIYNKDTLVIGVSERTNKEAILTIAEHIKNNKEAKFKKIVAINVPPMPNLMHLDTWLTMVDKNKFLYSPNMLSVLKIWEIDLSKEIKMVETSKPLADVLESIIGEKPILIPIAGENASQLDIDIETHFDGTNYLTIAPGVVVGYSRNVKTEAALKAAGVTVYSFDGNQLSLGMGSGRCMSMPLVREDVK

SEQ ID NO: 69 - protein, 281 aa, Homo sapiens [sequence omitted]

SEQ ID NO: 70 - protein, 168 aa, Homo sapiens
VRERGPQRVAAHITGTRGRSNTLSSPNSKNEKALGRKINSWESSRSGHSFLSNLHLRNGELVIHEKGFYYIYSQTYFRFQEEIKENTKNDKQMVQYIYKYTSYPDPILLMKSARNSCWSKDAEYGLYSIYQGGIFELKENDRIFVSVTNEHLIDMDHEASFFGAFLVG

SEQ ID NO: 71 - protein, 233 aa, Homo sapiens
MSTESMIRDVELAEEALPKKTGGPQGSRRCLFLSLFSFLIVAGATTLFCLLHFGVIGPQREEFPRDLSLISPLAQAVRSSSRTPSDKPVAHVVANPQAEGQLQWLNRRANALLANGVELRDNQLVVPSEGLYLIYSQVLFKGQGCPSTHVLLTHTISRIAVSYQTKVNLLSAIKSPCQRETPEGAEAKPWYEPIYLGGVFQLEKGDRLSAEINRPDYLDFAESGQVYFGIIAL

SEQ ID NO: 72 - protein, 281 aa, Homo sapiens
MQQPFNYPYPQIYWVDSSASSPWAPPGTVLPCPTSVPRRPGQRRPPPPPPPPPLPPPPPPPPLPPLPLPPLKKRGNHSTGLCLLVMFFMVLVALVGLGLGMFQLFHLQKELAELRESTSQMHTASSLEKQIGHPSPPPEKKELRKVAHLTGKSNSRSMPLEWEDTYGIVLLSGVKYKKGGLVINETGLYFVYSKVYFRGQSCNNLPLSHKVYMRNSKYPQDLVMMEGKMMSYCTTGQMWARSSYLGAVFNLTSADHLYVNVSELSLVNFEESQTFFGLYKL

SEQ ID NO: 73 - protein, 4 aa, Artificial Sequence
  Made in Lab - Linker
GSGS

SEQ ID NO: 74 - protein, 4 aa, Artificial Sequence
  Made in Lab - Linker
GGSG

SEQ ID NO: 75 - protein, 4 aa, Artificial Sequence
  Made in Lab - Linker
GGGS

SEQ ID NO: 76 - protein, 5 aa, Artificial Sequence
  Made in Lab - Linker
GGGGS

SEQ ID NO: 77 - protein, 4 aa, Artificial Sequence
  Made in Lab - Linker
GNGN

SEQ ID NO: 78 - protein, 4 aa, Artificial Sequence
  Made in Lab - Linker
GGNG

SEQ ID NO: 79 - protein, 4 aa, Artificial Sequence
  Made in Lab - Linker
GGGN

SEQ ID NO: 80 - protein, 5 aa, Artificial Sequence
  Made in Lab - Linker
GGGGN

SEQ ID NO: 81 - protein, 7 aa, Artificial Sequence
  Made in Lab - Linker
AEAAAKA

SEQ ID NO: 82 - protein, 12 aa, Artificial Sequence
  Made in Lab - Linker
AEAAAKEAAAKA

SEQ ID NO: 83 - protein, 6 aa, Artificial Sequence
  Made in Lab - Linker
APAPKP

SEQ ID NO: 84 - protein, 12 aa, Artificial Sequence
  Made in Lab - Linker
APAPKPEPAPKP

SEQ ID NO: 85 - protein, 10 aa, Artificial Sequence
  Made in Lab - Linker
GGGGSGGGGS

SEQ ID NO: 86 - protein, 5 aa, Artificial Sequence
  Made in Lab - Linker
DGGGS

SEQ ID NO: 87 - protein, 5 aa, Artificial Sequence
  Made in Lab - Linker
TGEKP

SEQ ID NO: 88 - protein, 4 aa, Artificial Sequence
  Made in Lab - Linker
GGRR

SEQ ID NO: 89 - protein, 14 aa, Artificial Sequence
  Made in Lab - Linker
EGKSSGSGSESKVD

SEQ ID NO: 90 - protein, 18 aa, Artificial Sequence
  Made in Lab - Linker
KESGSVSSEQLAQFRSLD

SEQ ID NO: 91 - protein, 8 aa, Artificial Sequence
  Made in Lab - Linker
GGRRGGGS

SEQ ID NO: 92 - protein, 9 aa, Artificial Sequence
  Made in Lab - Linker
LRQRDGERP

SEQ ID NO: 93 - protein, 12 aa, Artificial Sequence
  Made in Lab - Linker
LRQKDGGGSERP

SEQ ID NO: 94 - protein, 16 aa, Artificial Sequence
  Made in Lab - Linker
LRQKDGGGSGGGSERP

SEQ ID NO: 95 - DNA, 10 bp, Artificial Sequence
  Consensus Kozak sequence
rccrccatgg

SEQ ID NO: 96 - protein, 6 aa, Artificial Sequence
  Made in Lab - Linker
  MOD_RES (1)..(1): Xaa is any amino acid
  MOD_RES (3)..(3): Xaa is any amino acid
  MOD_RES (5)..(5): Xaa is any amino acid
XPXPXP

SEQ ID NO: 97 - protein, 12 aa, Artificial Sequence
  Made in Lab - Linker
  MOD_RES (1)..(1): Xaa is any amino acid
  MOD_RES (3)..(3): Xaa is any amino acid
  MOD_RES (5)..(5): Xaa is any amino acid
  MOD_RES (7)..(7): Xaa is any amino acid
  MOD_RES (9)..(9): Xaa is any amino acid
  MOD_RES (11)..(11): Xaa is any amino acid
XPXPXPXPXPXP